European Patent Application EP 4 495 242 A1, published January 22, 2025. Title: Antisense Nucleic Acid Inhibiting Chondroitin Sulfate Biosynthesis. Applicant: 学校法人　愛知医科大学. The sequence listing filed with the application follows.

SEQUENCE LISTING (41 sequences)

SEQ ID NO: 1 - DNA, 4299 bp, Homo sapiens
  source 1..4299: mol_type = genomic DNA
gttctccctggggagcgggaggctccaggcgcggctggggcgctgtgggcagatgcgctcggtcctcaccagcggcgttgtgcggcgaaccctgcggtgcttcgggaaggcggtcgttcctccctgctcccaccgttttccagcgtgtgcgctcttaccttctctggggaaaaaaggaaattttttattttttaacatttcatttcatgaaaccgttttttttaagtggtggcgctgaacacagtccttgcagaggggggcagcactttccctcctgaccccaacctggaaaccccagtgtgacttcagcgctgtcagagcattggaagcagagctgcgagttaggaagcggctcgctggcagctgggcacgtttctttcctgcgagatcggcttttttgatttgctctttttcacatgaaaatgttcagcttcatttttagacacctttagacatggttatcactgtttaaagccttgatttttttttaaacaaatagtttgcattttattcattgaaacagggagagaacaaataccatcctgctttttgggctgccttcctatttcaaggaaagacgccaaggtaattttgacccagaggagcaatgatgtagccacctcctaaccttcccttcttgaacccccagacataaagggagcagtaggcataaaatgtggggagctgaccatctgccggtccggtcctgaccttccactagtagtgagaccaatccagctcttgctgctgctgtggctttgtgaggaggtcccctcttgctgttggctgcacatcaggaaggctgtgatgggaatgaaggtgaaaacttggagatttcacttcagtcattgcttctgcctgcaagatcatcctttaaaagtagagaagctgctctgtgtggtggttaactccaagaggcagaactcgttctagaaggaaatggatgcaagcagctccgggggccccaaacgcatgcttcctgtggtctagcccagggaagcccttccgtgggggccccggctttgagggatgccaccggttctggacgcatggctgattcctgaatgatgatggttcgccgggggctgcttgcgtggatttcccgggtggtggttttgctggtgctcctctgctgtgctatctctgtcctgtacatgttggcctgcaccccaaaaggtgacgaggagcagctggcactgcccagggccaacagccccacggggaaggaggggtaccaggccgtccttcaggagtgggaggagcagcaccgcaactacgtgagcagcctgaagcggcagatcgcacagctcaaggaggagctgcaggagaggagtgagcagctcaggaatgggcagtaccaagccagcgatgctgctggcctgggtctggacaggagccccccagagaaaacccaggccgacctcctggccttcctgcactcgcaggtggacaaggcagaggtgaatgctggcgtcaagctggccacagagtatgcagcagtgcctttcgatagctttactctacagaaggtgtaccagctggagactggccttacccgccaccccgaggagaagcctgtgaggaaggacaagcgggatgagttggtggaagccattgaatcagccttggagaccctgaacagtcctgcagagaacagccccaatcaccgtccttacacggcctctgatttcatagaagggatctaccgaacagaaagggacaaagggacattgtatgagctcaccttcaaaggggaccacaaacacgaattcaaacggctcatcttatttcgaccattcggccccatcatgaaagtgaaaaatgaaaagctcaacatggccaacacgcttatcaatgttatcgtgcctctagcaaaaagggtggacaagttccggcagttcatgcagaatttcagggagatgtgcattgagcaggatgggagagtccatctcactgttgtttactttgggaaagaagaaataaatgaagtcaaaggaatacttgaaaacacttccaaagctgccaacttcaggaactttaccttcatccagctgaatggagaattttctcggggaaagggacttgatgttggagcccgcttctggaagggaagcaacgtccttctctttttctgtgatgtggacatctacttcacatctgaattcctcaatacgtgtaggctgaatacacagccagggaagaaggtattttatccagttcttttcagtcagtacaatcctggcataatatacggccaccatgatgcagtccctcccttggaacagcagctggtcataaagaaggaaactggattttggagagactttggatttgggatgacgtgtcagtatcggtcagacttcatcaatataggtgggtttgatctggacatcaaaggctggggcggagaggatgtgcacctttatcgcaagtatctccacagcaacctcatagtggtacggacgcctgtgcgaggactcttccacctctggcatgagaagcgctgcatggacgagctgacccccgagcagtacaagatgtgcatgcagtccaaggccatgaacgaggcatcccacggccagctgggcatgctggtgttcaggcacgagatagaggctcaccttcgcaaacagaaacagaagacaagtagcaaaaaaacatgaactcccagagaaggattgtgggagacactttttctttccttttgcaattactgaaagtggctgcaacagagaaaagacttccataaaggacgacaaaagaattggactgatgggtcagagatgagaaagcctccgatttctctctgttgggctttttacaacagaaatcaaaatctccgctttgcctgcaaaagtaacccagttgcaccctgtgaagtgtctgacaaaggcagaatgcttgtgagattataagcctaatggtgtggaggttttgatggtgtttacaacacactgagacctgttgttttgtgtgctcattgaaatattcatgatttaagagcagttttgtaaaaaattcattagcatgaaaggcaagcatatttctcctcatatgaatgagcctatcagcagggctctagtttctaggaatgctaaaatatcagaaggcaggagaggagataggcttattatgatactagtgagtacattaagtaaaataaaatggaccagaaaagaaaagaaaccataaatatcgtgtcatattttccccaagattaaccaaaaataatctgcttatctttttggttgtccttttaactgtctccgtttttttcttttatttaaaaatgcactttttttcccttgtgagttatagtctgcttatttaattaccactttgcaagccttacaagagagcacaagttggcctacatttttatattttttaagaagatactttgagatgcattatgagaactttcagttcaaagcatcaaattgatgccatatccaaggacatgccaaatgctgattctgtcaggcactgaatgtcaggcattgagacatagggaaggaatggtttgtactaatacagacgtacagatactttctctgaagagtattttcgaagaggagcaactgaacactggaggaaaagaaaatgacactttctgctttacagaaaaggaaactcattcagactggtgatatcgtgatgtacctaaaagtcagaaaccacattttctcctcagaagtagggaccgctttcttacctgtttaaataaaccaaagtataccgtgtgaaccaaacaatctcttttcaaaacagggtgctcctcctggcttctggcttccataagaagaaatggagaaaaaaatatatatatatatattgtgaaagatcaatccatctgccagaatctagtgggatggaagtttttgctacatgttatccaccccaggccaggtggaagtaactgaattattttttaaattaagcagttctactcgatcaccaagatgcttctgaaaattgcattttattaccatttcaaactattttttaaaaataaatacagttaacatagagtggtttcttcattcatgtgaaaattattagccagcaccagatgcatgagctaattatctctttgagtccttgcttctgtttgctcacagtaaactcattgtttaaaagcttcaagaacattcaagctgttggtgtgttaaaaaatgcattgtattgatttgtactggtagtttatgaaatttaattaaaacacaggccatgaatggaaggtggtattgcacagctaataaaatatgatttgtggatatgaaaaaaaaaaaaaaaaaa

SEQ ID NO: 2 - DNA, 15 bp, synthetic construct
  misc_feature 1..15: note = anti-sense nucleotide_LX-A1011, 2957
  source 1..15: mol_type = other DNA
ctgcatactctgtgg

SEQ ID NO: 3 - DNA, 15 bp, synthetic construct
  misc_feature 1..15: note = anti-sense nucleotide_LX-A1012
  source 1..15: mol_type = other DNA
gctgcatactctgtg

SEQ ID NO: 4 - DNA, 15 bp, synthetic construct
  misc_feature 1..15: note = anti-sense nucleotide_LX-A1013
  source 1..15: mol_type = other DNA
tgctgcatactctgt

SEQ ID NO: 5 - DNA, 15 bp, synthetic construct
  misc_feature 1..15: note = anti-sense nucleotide_LX-A1016
  source 1..15: mol_type = other DNA
agagtaaagctatcg

SEQ ID NO: 6 - DNA, 15 bp, synthetic construct
  misc_feature 1..15: note = anti-sense nucleotide_LX-A1017
  source 1..15: mol_type = other DNA
tagagtaaagctatc

SEQ ID NO: 7 - DNA, 15 bp, synthetic construct
  misc_feature 1..15: note = anti-sense nucleotide_LX-A1018
  source 1..15: mol_type = other DNA
gtagagtaaagctat

SEQ ID NO: 8 - DNA, 15 bp, synthetic construct
  misc_feature 1..15: note = anti-sense nucleotide_LX-A1019
  source 1..15: mol_type = other DNA
tgtagagtaaagcta

SEQ ID NO: 9 - DNA, 15 bp, synthetic construct
  misc_feature 1..15: note = anti-sense nucleotide_LX-A1028
  source 1..15: mol_type = other DNA
aggctgattcaatgg

SEQ ID NO: 10 - DNA, 15 bp, synthetic construct
  misc_feature 1..15: note = anti-sense nucleotide_LX-A1029
  source 1..15: mol_type = other DNA
ccaaggctgattcaa

SEQ ID NO: 11 - DNA, 15 bp, synthetic construct
  misc_feature 1..15: note = anti-sense nucleotide_LX-A1045, 1885, 1886
  source 1..15: mol_type = other DNA
aacattgataagcgt

SEQ ID NO: 12 - DNA, 15 bp, synthetic construct
  misc_feature 1..15: note = anti-sense nucleotide_LX-A1046
  source 1..15: mol_type = other DNA
taacattgataagcg

SEQ ID NO: 13 - DNA, 15 bp, synthetic construct
  misc_feature 1..15: note = anti-sense nucleotide_LX-A1047, 1887, 1888
  source 1..15: mol_type = other DNA
ataacattgataagc

SEQ ID NO: 14 - DNA, 15 bp, synthetic construct
  misc_feature 1..15: note = anti-sense nucleotide_LX-A1048
  source 1..15: mol_type = other DNA
cgataacattgataa

SEQ ID NO: 15 - DNA, 15 bp, synthetic construct
  misc_feature 1..15: note = anti-sense nucleotide_LX-A1054
  source 1..15: mol_type = other DNA
ttttgctagaggcac

SEQ ID NO: 16 - DNA, 15 bp, synthetic construct
  misc_feature 1..15: note = anti-sense nucleotide_LX-A1076
  source 1..15: mol_type = other DNA
ggattgtactgactg

SEQ ID NO: 17 - DNA, 15 bp, synthetic construct
  misc_feature 1..15: note = anti-sense nucleotide_LX-A1077
  source 1..15: mol_type = other DNA
aggattgtactgact

SEQ ID NO: 18 - DNA, 15 bp, synthetic construct
  misc_feature 1..15: note = anti-sense nucleotide_LX-A1078
  source 1..15: mol_type = other DNA
caggattgtactgac

SEQ ID NO: 19 - DNA, 15 bp, synthetic construct
  misc_feature 1..15: note = anti-sense nucleotide_LX-A1079
  source 1..15: mol_type = other DNA
ccaggattgtactga

SEQ ID NO: 20 - DNA, 15 bp, synthetic construct
  misc_feature 1..15: note = anti-sense nucleotide_LX-A1080
  source 1..15: mol_type = other DNA
tgccaggattgtact

SEQ ID NO: 21 - DNA, 15 bp, synthetic construct
  misc_feature 1..15: note = anti-sense nucleotide_LX-A1090
  source 1..15: mol_type = other DNA
acgtcatcccaaatc

SEQ ID NO: 22 - DNA, 15 bp, synthetic construct
  misc_feature 1..15: note = anti-sense nucleotide_LX-A1091
  source 1..15: mol_type = other DNA
cacgtcatcccaaat

SEQ ID NO: 23 - DNA, 15 bp, synthetic construct
  misc_feature 1..15: note = anti-sense nucleotide_LX-A1101
  source 1..15: mol_type = other DNA
accactatgaggttg

SEQ ID NO: 24 - DNA, 15 bp, synthetic construct
  misc_feature 1..15: note = anti-sense nucleotide_LX-A1191, 2996
  source 1..15: mol_type = other DNA
gattgtttggttcac

SEQ ID NO: 25 - DNA, 15 bp, synthetic construct
  misc_feature 1..15: note = anti-sense nucleotide_LX-A1192, 2962
  source 1..15: mol_type = other DNA
agattgtttggttca

SEQ ID NO: 26 - DNA, 15 bp, synthetic construct
  misc_feature 1..15: note = anti-sense nucleotide_LX-A1193, 1899, 1900
  source 1..15: mol_type = other DNA
gagattgtttggttc

SEQ ID NO: 27 - DNA, 15 bp, synthetic construct
  misc_feature 1..15: note = anti-sense nucleotide_LX-A1897, 1898
  source 1..15: mol_type = other DNA
gattgtttggttcac

SEQ ID NO: 28 - DNA, 15 bp, synthetic construct
  misc_feature 1..15: note = anti-sense nucleotide_LX-A1901, 1902
  source 1..15: mol_type = other DNA
gtaccactatgaggt

SEQ ID NO: 29 - DNA, 17 bp, synthetic construct
  misc_feature 1..17: note = anti-sense nucleotide_LX-A2997
  source 1..17: mol_type = other DNA
gagattgtttggttcac

SEQ ID NO: 30 - DNA, 17 bp, synthetic construct
  misc_feature 1..17: note = anti-sense nucleotide_LX-A2998
  source 1..17: mol_type = other DNA
ctgcatactctgtggcc

SEQ ID NO: 31 - DNA, 17 bp, synthetic construct
  misc_feature 1..17: note = anti-sense nucleotide_LX-A2999
  source 1..17: mol_type = other DNA
cacgtcatcccaaatcc

SEQ ID NO: 32 - DNA, 15 bp, synthetic construct
  misc_feature 1..15: note = Negative Control
  source 1..15: mol_type = other DNA
gaaaactaaaatgag

SEQ ID NO: 33 - DNA, 15 bp, synthetic construct
  misc_feature 1..15: note = anti-sense nucleotide_LX-A1357
  source 1..15: mol_type = other DNA
acatcacagaaaaag

SEQ ID NO: 34 - DNA, 20 bp, synthetic construct
  misc_feature 1..20: note = Primer
  source 1..20: mol_type = other DNA
tcagggagatgtgcattgag

SEQ ID NO: 35 - DNA, 20 bp, synthetic construct
  misc_feature 1..20: note = Primer
  source 1..20: mol_type = other DNA
agttggcagctttggaagtg

SEQ ID NO: 36 - DNA, 20 bp, synthetic construct
  misc_feature 1..20: note = Primer
  source 1..20: mol_type = other DNA
ggagaccctgaacagtcctg

SEQ ID NO: 37 - DNA, 20 bp, synthetic construct
  misc_feature 1..20: note = Primer
  source 1..20: mol_type = other DNA
gccgtttgaattcgtgtttg

SEQ ID NO: 38 - DNA, 20 bp, synthetic construct
  misc_feature 1..20: note = Primer
  source 1..20: mol_type = other DNA
gagtcaacggatttggtcgt

SEQ ID NO: 39 - DNA, 20 bp, synthetic construct
  misc_feature 1..20: note = Primer
  source 1..20: mol_type = other DNA
gacaagcttcccgttctcag

SEQ ID NO: 40 - DNA, 16 bp, synthetic construct
  misc_feature 1..16: note = anti-sense nucleotide_PC1
  source 1..16: mol_type = other DNA
atcatggctgcagctt

SEQ ID NO: 41 - DNA, 15 bp, synthetic construct
  misc_feature 1..15: note = anti-sense nucleotide_PC2
  source 1..15: mol_type = other DNA
gtcatcccaaatcca